European Patent Application EP 4 585 588 A1, published July 16, 2025. Title: 一种苯并咪唑类化合物及其制备方法和应用. Applicant: 苏州沪云新药研发股份有限公司. The sequence listing filed with the application follows.

SEQUENCE LISTING (4 sequences)

SEQ ID NO: 1 - DNA, 20 bp, synthetic construct
  source 1..20: mol_type = other DNA
agagacggcagtgctctagg

SEQ ID NO: 2 - DNA, 20 bp, synthetic construct
  source 1..20: mol_type = other DNA
caatcctacccccgaagcag

SEQ ID NO: 3 - DNA, 20 bp, synthetic construct
  source 1..20: mol_type = other DNA
ctccaggggtgatggacaac

SEQ ID NO: 4 - DNA, 20 bp, synthetic construct
  source 1..20: mol_type = other DNA
cgatacctctgccggaagtc